European Patent Specification EP 3 296 393 B1, published March 4, 2026. Title: Method for producing cell culture comprising megakaryocytes and platelets with the cell culture. Applicant: Megakaryon Corporation. The sequence listing filed with the application follows.

SEQUENCE LISTING (1 sequence)

SEQ ID NO: 1 - DNA, 948 bp, Homo sapiens
tgtgaacggaccaagagtaaacagtgtgctcaatgctgtgcctacgtgtgttagcccacgcggccagcctgaggagtcagggaaggctcccctaggcaaagcccccaaccagaatcaagtcttaatggttaaagagctccatcacccaaaaaggattgagggcctaccttcaactgaacagctaatgcataatctcagaaactgtgagtcaaaattccctggaataactccactttatccccaatctccttgccacctagaccaaggtccattcaccaccctgtccccagcactgactgcactgctgtggccacactaaagcttggctcaagacggaggaggagtgaggaagctgctgcaccaatatggctggttgaggccgcccaaggtcctagaaggaggaagtgggtaaatgccatatccaaaaagatacagaagcctcaggttttatcgggggcagcagcttccttctccttccccgacctgtggccaagtcacaaagcaccacagctgtacagccagatgggggaagggaggagattagaactgtaggctagagtagacaagtatggaccagttcacaatcacgctatcccaagcagaaagtgatggtggcttggactagcacggtggtagtagagatggggtaaagattcaagagacatcattgataggcagaaccaataggacatggtaataaactattctcaggaaaggggaggagtcatggctttcagccatgagcatccaccctctgggtggcctcacccacttcctggcaattctagccaccatgagtccaggggctatagccctttgctctgcccgttgctcagcaagttacttggggttccagtttgataagaaaagacttcctgtggaggaatctgaagggaaggaggaggagctggcccattcctgcctgggaggttgtggaagaaggaagat